European Patent Application EP 4 209 591 A1, published July 12, 2023. Title: METHOD FOR PREPARING NON-HUMAN MAMMAL OR PROGENY THEREOF, AND USE THEREOF. Applicant: RenGene Biotechnology Co., Ltd. Application EP21863668.6. The sequence listing filed with the application follows.

SEQUENCE LISTING (76 sequences)

SEQ ID NO: 1 - DNA, 20 bp, Mus musculus
  misc_feature (1)..(20): Targeting sequence for sgRNA selected on the upstream portion of the first exon of the Ighm gene in the mouse
gactctctgaggaccagaga

SEQ ID NO: 2 - DNA, 20 bp, Mus musculus
  misc_feature (1)..(20): Targeting sequence for sgRNA selected on the upstream portion of the first exon of the Ighm gene in the mouse
tgggaaggactgactctctg

SEQ ID NO: 3 - DNA, 20 bp, Mus musculus
  misc_feature (1)..(20): Targeting sequence for sgRNA selected on the downstream portion of the first exon of the Ighg2c gene in the mouse
agtggacaagaaaattggtg

SEQ ID NO: 4 - DNA, 20 bp, Mus musculus
  misc_feature (1)..(20): Targeting sequence for sgRNA selected on the downstream portion of the first exon of the Ighg2c gene in the mouse
cttgtgaacttctactcccc

SEQ ID NO: 5 - DNA, 20 bp, Mus musculus
  misc_feature (1)..(20): Targeting sequence for sgRNA selected on the downstream portion of the first exon of the Ighm gene in the mouse
gatctgcatgtgcccattcc

SEQ ID NO: 6 - DNA, 20 bp, Mus musculus
  misc_feature (1)..(20): Targeting sequence for sgRNA selected on the downstream portion of the first exon of the Ighm gene in the mouse
ggtttggttcttacctggaa

SEQ ID NO: 7 - DNA, 20 bp, Mus musculus
  misc_feature (1)..(20): Targeting sequence for sgRNA selected on the upstream portion of the first exon of the Ighg3 gene in the mouse
tgttgtagctgcaagatagg

SEQ ID NO: 8 - DNA, 20 bp, Mus musculus
  misc_feature (1)..(20): Targeting sequence for sgRNA selected on the upstream portion of the first exon of the Ighg3 gene in the mouse
gagtgaggttatcagacagc

SEQ ID NO: 9 - RNA, 113 nt, Artificial sequence
  misc_feature (1)..(113): sgRNA sequence targeting the upstream portion of the first exon of the Ighm gene in the mouse
gacucucugaggaccagagaguuuaagagcuaugcuggaaacagcauagcaaguuuaaauaaggcuaguccguuaucaacuugaaaaaguggcaccgagucggugcuuuuuuu

SEQ ID NO: 10 - RNA, 114 nt, Artificial sequence
  misc_feature (1)..(114): sgRNA sequence targeting the upstream portion of the first exon of the Ighm gene in the mouse
gugggaaggacugacucucugguuuaagagcuaugcuggaaacagcauagcaaguuuaaauaaggcuaguccguuaucaacuugaaaaaguggcaccgagucggugcuuuuuuu

SEQ ID NO: 11 - RNA, 114 nt, Artificial sequence
  misc_feature (1)..(114): sgRNA sequence targeting the downstream portion of the first exon of the Ighg2c gene in the mouse
gaguggacaagaaaauuggugguuuaagagcuaugcuggaaacagcauagcaaguuuaaauaaggcuaguccguuaucaacuugaaaaaguggcaccgagucggugcuuuuuuu

SEQ ID NO: 12 - RNA, 114 nt, Artificial sequence
  misc_feature (1)..(114): sgRNA sequence targeting the downstream portion of the first exon of the Ighg2c gene in the mouse
gcuugugaacuucuacuccccguuuaagagcuaugcuggaaacagcauagcaaguuuaaauaaggcuaguccguuaucaacuugaaaaaguggcaccgagucggugcuuuuuuu

SEQ ID NO: 13 - RNA, 113 nt, Artificial sequence
  misc_feature (1)..(113): sgRNA sequence targeting the downstream portion of the first exon of the Ighm gene in the mouse
gaucugcaugugcccauuccguuuaagagcuaugcuggaaacagcauagcaaguuuaaauaaggcuaguccguuaucaacuugaaaaaguggcaccgagucggugcuuuuuuu

SEQ ID NO: 14 - RNA, 113 nt, Artificial sequence
  misc_feature (1)..(113): sgRNA sequence targeting the downstream portion of the first exon of the Ighm gene in the mouse
gguuugguucuuaccuggaaguuuaagagcuaugcuggaaacagcauagcaaguuuaaauaaggcuaguccguuaucaacuugaaaaaguggcaccgagucggugcuuuuuuu

SEQ ID NO: 15 - RNA, 114 nt, Artificial sequence
  misc_feature (1)..(114): sgRNA sequence targeting the upstream portion of the first exon of the Ighg3 gene in the mouse
guguuguagcugcaagauaggguuuaagagcuaugcuggaaacagcauagcaaguuuaaauaaggcuaguccguuaucaacuugaaaaaguggcaccgagucggugcuuuuuuu

SEQ ID NO: 16 - RNA, 113 nt, Artificial sequence
  misc_feature (1)..(113): sgRNA sequence targeting the upstream portion of the first exon of the Ighg3 gene in the mouse
gagugagguuaucagacagcguuuaagagcuaugcuggaaacagcauagcaaguuuaaauaaggcuaguccguuaucaacuugaaaaaguggcaccgagucggugcuuuuuuu

SEQ ID NO: 17 - DNA, 20 bp, Artificial sequence
  misc_feature (1)..(20): PCR primer Ighm-d-g-1F, capable of detecting the genes which are knocked out
gttcatgcccctagagttgg

SEQ ID NO: 18 - DNA, 20 bp, Artificial sequence
  misc_feature (1)..(20): PCR primer Ighm-d-g-1R, capable of detecting the genes which are knocked out
taccattctccctggagtgg

SEQ ID NO: 19 - DNA, 20 bp, Artificial sequence
  misc_feature (1)..(20): PCR primer Ighd-2F, capable of detecting wild-type genes
gctcctgagactggccatag

SEQ ID NO: 20 - DNA, 20 bp, Artificial sequence
  misc_feature (1)..(20): PCR primer Ighd-2R, capable of detecting wild-type genes
aaaagggagggaatgaatgg

SEQ ID NO: 21 - DNA, 27 bp, Artificial sequence
  misc_feature (1)..(27): PCR primer MHV1
  misc_feature (21)..(21): s=g or c
atgaaatgcagctggggcatsttcttc

SEQ ID NO: 22 - DNA, 26 bp, Artificial sequence
  misc_feature (1)..(26): PCR primer MHV2
  misc_feature (14)..(14): r=g or a
  misc_feature (21)..(21): s=g or c
  misc_feature (22)..(22): y=t or c
atgggatggagctrtatcatsytctt

SEQ ID NO: 23 - DNA, 27 bp, Artificial sequence
  misc_feature (1)..(27): PCR primer MHV3
  misc_feature (7)..(7): w=a or t
atgaagwtgtggttaaactgggttttt

SEQ ID NO: 24 - DNA, 25 bp, Artificial sequence
  misc_feature (1)..(25): PCR primer MHV4
  misc_feature (4)..(4): r=g or a
  misc_feature (13)..(13): y=t or c
  misc_feature (22)..(22): r=g or a
atgractttgggytcagcttgrttt

SEQ ID NO: 25 - DNA, 32 bp, Artificial sequence
  misc_feature (1)..(32): PCR primer MHV5
atgggactccaggcttcaatttagttttcctt

SEQ ID NO: 26 - DNA, 29 bp, Artificial sequence
  misc_feature (1)..(29): PCR primer MHV6
  misc_feature (11)..(11): y=t or c
  misc_feature (14)..(14): r=g or a
  misc_feature (16)..(16): s=g or c
  misc_feature (20)..(20): r=g or a
atggcttgtcyttrgsgctrctcttctgc

SEQ ID NO: 27 - DNA, 27 bp, Artificial sequence
  misc_feature (1)..(27): PCR primer MHV7
  misc_feature (5)..(5): r=g or a
  misc_feature (13)..(13): k=g or t
  misc_feature (16)..(16): r=g or a
  misc_feature (23)..(23): m=a or c
atggratggagckggrgtctttmtctt

SEQ ID NO: 28 - DNA, 23 bp, Artificial sequence
  misc_feature (1)..(23): PCR primer MHV8
atgagagtgctgattcttttgtg

SEQ ID NO: 29 - DNA, 31 bp, Artificial sequence
  misc_feature (1)..(31): PCR primer MHV9
  misc_feature (5)..(5): m=a or c
  misc_feature (17)..(17): m=a or c
atggmttgggtgtggamcttgcttattcctg

SEQ ID NO: 30 - DNA, 28 bp, Artificial sequence
  misc_feature (1)..(28): PCR primer MHV10
atgggcagacttaccattctcattcctg

SEQ ID NO: 31 - DNA, 28 bp, Artificial sequence
  misc_feature (1)..(28): PCR primer MHV11
atggattttgggctgattttttttattg

SEQ ID NO: 32 - DNA, 26 bp, Artificial sequence
  misc_feature (1)..(26): PCR primer MHV12
atgatggtgttaagtccttctgtacc

SEQ ID NO: 33 - DNA, 20 bp, Artificial sequence
  misc_feature (1)..(20): PCR primer B6_IgG2c_CH2 R1
tggtccacccaagaggtctg

SEQ ID NO: 34 - DNA, 49 bp, Artificial sequence
  misc_feature (1)..(41): PCR primer MHVF1-SfiI
atgccatgactgtggcccaggcggccgaggtgaagcttctcgagtctgg

SEQ ID NO: 35 - DNA, 50 bp, Artificial sequence
  misc_feature (1)..(42): PCR primer MHVF2-SfiI
  misc_feature (28)..(28): s=g or c
  misc_feature (33)..(33): s=g or c
  misc_feature (40)..(40): m=a or c
  misc_feature (48)..(48): w=a or t
catgccatgactgtggcccaggcggccsaggtscagctgmaggagtcwgg

SEQ ID NO: 36 - DNA, 50 bp, Artificial sequence
  misc_feature (1)..(42): PCR primer MHVF3-SfiI
catgccatgactgtggcccaggcggccgaggtccagctgcaacaatctgg

SEQ ID NO: 37 - DNA, 50 bp, Artificial sequence
  misc_feature (1)..(42): PCR primer MHVF4-SfiI
  misc_feature (28)..(28): s=g or c
  misc_feature (33)..(33): y=t or c
  misc_feature (36)..(36): r=g or a
  misc_feature (39)..(39): k=g or t
  misc_feature (46)..(46): y=t or c
catgccatgactgtggcccaggcggccsaggtycarctkcagcagyctgg

SEQ ID NO: 38 - DNA, 50 bp, Artificial sequence
  misc_feature (1)..(41): PCR primer MHVF5-SfiI
  misc_feature (30)..(30): r=g or a
  misc_feature (41)..(41): w=a or t
catgccatgactgtggcccaggcggccgargtgaagcttgwggagtctgg

SEQ ID NO: 39 - DNA, 37 bp, Artificial sequence
  misc_feature (1)..(37): PCR primer B6-IgG2c-Hin-sfi1
actcgcggccggcctggcctgttatgggcactctggg

SEQ ID NO: 40 - DNA, 357 bp, Mus musculus
  misc_feature (1)..(357): Nucleotide sequence of CRP antigen-specific IgG2c heavy chain antibody variable region
gaggtccagctgcaacaatctggacctgagttggtgaagcctggggcttcagtgaagatttcctgtaaggcttctggatacatgttcagtgactactatatgaattgggtgaagcagagccatggaaagagccttgagtggattggaaatgttgatcctaacactgataatactatatacaaccagaacttcaaggacaaggccacattgactgtagacaggtcctccagaacagcctacatggaactccacagcctgacatctgaggactctgcagtctattactgtgcaagatcgaggttctatgatccctggtttgcttactggggccaagggactctggtcactgtctctgca

SEQ ID NO: 41 - protein, 119 aa, Mus musculus
  DOMAIN (1)..(119): Amino acid sequence of CRP antigen-specific IgG2c heavy chain antibody variable region
EVQLQQSGPELVKPGASVKISCKASGYMFSDYYMNWVKQSHGKSLEWIGNVDPNTDNTIYNQNFKDKATLTVDRSSRTAYMELHSLTSEDSAVYYCARSRFYDPWFAYWGQGTLVTVSA

SEQ ID NO: 42 - DNA, 348 bp, Mus musculus
  misc_feature (1)..(348): Nucleotide sequence of CRP antigen-specific IgG2c heavy chain antibody variable region
gaggtgaagcttctcgagtctgggggaggcttagtgaagcctggagggtccctgaaactctcctgtgcagcctctggattcactttcagtgactatggcatgtcttggattcgccagactccagacaagaggctggagtgggtcgcaaccattagtagtggtaatacttacacctattattcaaaaagtgtgaaggggcgattcaccatctccagagacaatgccaagaacaccctgtacctgcaaatgagcagtctgaagtctgaagacacagccatatattactgttcaagacatacctctgattattaccctctgagccaagggactctggtcactgtctctgca

SEQ ID NO: 43 - protein, 116 aa, Mus musculus
  DOMAIN (1)..(116): Amino acid sequence of CRP antigen-specific IgG2c heavy chain antibody variable region
EVKLLESGGGLVKPGGSLKLSCAASGFTFSDYGMSWIRQTPDKRLEWVATISSGNTYTYYSKSVKGRFTISRDNAKNTLYLQMSSLKSEDTAIYYCSRHTSDYYPLSQGTLVTVSA

SEQ ID NO: 44 - DNA, 20 bp, Artificial sequence
  misc_feature (1)..(20): PCR primer Ighm-F, capable of detecting the genes which are knocked out
ctgtggctagaaggcagctc

SEQ ID NO: 45 - DNA, 20 bp, Artificial sequence
  misc_feature (1)..(20): PCR primer Ighm-R, capable of detecting the genes which are knocked out
atctctgcgacagctggaat

SEQ ID NO: 46 - DNA, 18 bp, Artificial sequence
  misc_feature (1)..(18): PCR primer B6- IghM CH2 R4
gttcatctctgcgacagc

SEQ ID NO: 47 - protein, 117 aa, Mus musculus
  DOMAIN (1)..(117): Amino acid sequence of CRP antigen-specific IgG2c heavy chain antibody variable region
EVQLQQSGPEVLKPGTSVRMSCKASGYTFTDYNIHWVKQSRGESLEWIGFVNPDTGDTYYYKNFKGKATLTFNRSSSTAYMDLRSLTSEDSAVYYCARGTTVEKDYWGQGTILTVSS

SEQ ID NO: 48 - protein, 117 aa, Mus musculus
  DOMAIN (1)..(117): Amino acid sequence of CRP antigen-specific IgG2c heavy chain antibody variable region
EVQLQQSGPELVKPGASVRMSCKASGYTFTDYNIHWVKQSHGESLEWIGFVNPDNGDTYYYKNFKGKATLTFNRSSSTAYMDLRSLTSEDSAVYYCARGTTVEKDYWGQGTTLTVSS

SEQ ID NO: 49 - protein, 117 aa, Mus musculus
  DOMAIN (1)..(117): Amino acid sequence of CRP antigen-specific IgG2c heavy chain antibody variable region
EVQLQQSGPELVKPGASVRMSCKASGYTFTDYNIHWVKQSHGESLEWIGFINPDNGDTYYYKNFRGKATLTLNKSSSTAYMDLRSLTSEDSGVYYCARGTTVEKDYWGQGTILTVSS

SEQ ID NO: 50 - protein, 124 aa, Mus musculus
  DOMAIN (1)..(124): Amino acid sequence of coronavirus S protein antigen-specific IgG2c heavy chain antibody S-9 variable region
EVQLQQSGPELVKPGASVKISCKASGYTFTDYYMNWVKQSHGKSLEWIGDINPNNGDANYNQSFKGKATLTVDKSSSTAYMELRSLTSEDSAVYYCAKPPLYYYNDSHWYFNVWGTGTTVTVSS

SEQ ID NO: 51 - protein, 124 aa, Mus musculus
  DOMAIN (1)..(124): Amino acid sequence of coronavirus S protein antigen-specific IgG2c heavy chain antibody S-19 variable region
EVQLQQSGPELVKPGASVKISCKASGYTFTDYYMNWVKQSHGKSLEWIGDINPNNSDSNYNQNFKDKATLTVDRSSSTAYMELRSLTSEDSAVYYCAKPPLYYYNNSHWYFNVWGTGTTVTVSS

SEQ ID NO: 52 - protein, 124 aa, Mus musculus
  DOMAIN (1)..(124): Amino acid sequence of coronavirus S protein antigen-specific IgG2c heavy chain antibody S-27 variable region
EVQLQQSGPELVKPGASVKISCKASGYTFTDYYMNWVKQSHGRSLEWIGDINPNNGDTNYNPNFKDKATLTVDMSSTTAYMELRSLTSEDSAVYFCAKPPLYYYNNSHWYFNVWGTGTTVTVSS

SEQ ID NO: 53 - protein, 116 aa, Mus musculus
  DOMAIN (1)..(116): Amino acid sequence of coronavirus S protein antigen-specific IgG2c heavy chain antibody S-47 variable region
EVQLQQSGPELVKPGDSVKISCKASGYSFTDYFINWVMRSHGKGLEWIGRINPYNGDTFFNQKFKGKAILTVDTSSSTAHMELRSLTSEDSAVYYCATYGSPMDYWGQGTSVTVSS

SEQ ID NO: 54 - protein, 124 aa, Mus musculus
  DOMAIN (1)..(124): Amino acid sequence of coronavirus S protein antigen-specific IgG2c heavy chain antibody S-1 variable region
EVQLQQSGPELVKPGASVKISCKASGYTFTDYYMNWVKQSHGKSLEWIGDINPNNGGANYNQTFKGKATFTVDKSSSTAYMELRSLTSEDSAVYYCAKGPLYYYNSSNWYFDVRGTGTTVTVSS

SEQ ID NO: 55 - protein, 124 aa, Mus musculus
  DOMAIN (1)..(124): Amino acid sequence of coronavirus S protein antigen-specific IgG2c heavy chain antibody S-2 variable region
EVQLQQSGPELVKPGASVKISCKASGYTFTDYYMNWVKQSHGKSLEWIGDINPNNGGTSYNQKFKGKATLTVDKSSSTAYMELRSLTSEDSAVYYCAKGPLYYYNSSNWYFDVRGTGTTVTVSS

SEQ ID NO: 56 - protein, 124 aa, Mus musculus
  DOMAIN (1)..(124): Amino acid sequence of coronavirus S protein antigen-specific IgG2c heavy chain antibody S-7 variable region
EVQLQQSGPELVKPGASVKISCKASGYTFTDYYINWVKQSHGKSREWIGDINPKNGGTNFNREFKGEATLTVDKSSTTAYMELRSLTSEDSAVYYCAKGPLYYYNNSYWYFDVWGTGTTVTVSS

SEQ ID NO: 57 - protein, 124 aa, Mus musculus
  DOMAIN (1)..(124): Amino acid sequence of coronavirus S protein antigen-specific IgG2c heavy chain antibody S-12 variable region
EVQLQQSGPELVKPGASVKISCKASGYTFTDYYMNWVKQSHGKSREWIGDINPNNGVTSYNQNFKGEATLTVDKSSSTAYMELRSLTSEDSAVYYCAKGPLYYYNSSNWYFDVWGTGTTVTVSS

SEQ ID NO: 58 - protein, 124 aa, Mus musculus
  DOMAIN (1)..(124): Amino acid sequence of coronavirus S protein antigen-specific IgG2c heavy chain antibody S-17 variable region
EVQLQQSGPELVKPGASVKISCKASGYMFTDYYMNWVKQSHGKSLEWIGDINPNNGGANYNQKFKGKATLTVDKSSSTAYMELRSLTSEDSAVYYCAKGPLYYYNSSNWYFDVRGTGTTVTVSS

SEQ ID NO: 59 - protein, 124 aa, Mus musculus
  DOMAIN (1)..(124): Amino acid sequence of coronavirus S protein antigen-specific IgG2c heavy chain antibody S-19 variable region
EVQLQQSGPELVKPGASVKISCKASGYTFTDYYMNWVKQSHGKSLEWIGDINPNNGGANYNQTFKGKATLTVDKSSSTAYMELRSLTSEDSAVYYCAKGPLYYYNSSTWYFDVRGTGTTVTVSS

SEQ ID NO: 60 - protein, 124 aa, Mus musculus
  DOMAIN (1)..(124): Amino acid sequence of coronavirus S protein antigen-specific IgG2c heavy chain antibody S-25 variable region
EVQLQQSGPELVKPGASVKISCKASGYTFTDYYMNWVKQSHGKSLEWIGDINPNNGGTSYNQKFKGKATLTVDKSSSTAYMELRSLTSEDSAVYYCAKGPLYYYNNSNWYFDVRGTGTTVTVSS

SEQ ID NO: 61 - protein, 124 aa, Mus musculus
  DOMAIN (1)..(124): Amino acid sequence of coronavirus S protein antigen-specific IgG2c heavy chain antibody S-51 variable region
EVQLQQSGPELVKPGASVKISCKASGYTFTDYYMNWVKQSHGKSLEWIGDINPSTGGTSYNQTFKGKATLTVDKSSSTAYMELRSLTSEDSAVYYCAKGPLYYYNSSNWYFDVRGTGTTVTVSS

SEQ ID NO: 62 - protein, 124 aa, Mus musculus
  DOMAIN (1)..(124): Amino acid sequence of coronavirus S protein antigen-specific IgG2c heavy chain antibody S-65 variable region
EVQLQQSGPELVKPGASVKISCKASGYTFTDYYINWVKQSHGKSLEWIGDINPKNGGSNYNQTFKGEATLTVDKSSNTAYMELRSLTSEDSAVYYCARGPLYYYNSTYWYFDVWGTGTTVTVSS

SEQ ID NO: 63 - protein, 122 aa, Mus musculus
  DOMAIN (1)..(122): Amino acid sequence of coronavirus N protein antigen-specific IgG2c heavy chain antibody N-1 variable region
EVQLQESGPGMVKPSQSLSLTCTVTGYSITSGYDWHWIRQFPGNKQEWLGYITYDGSNHYNPSLKNRISITRDTSKNQFFLKLSSVTTEDTATYYCARGDDYDGDYYTMDYWGQGTSVTVSS

SEQ ID NO: 64 - protein, 122 aa, Mus musculus
  DOMAIN (1)..(122): Amino acid sequence of coronavirus N protein antigen-specific IgG2c heavy chain antibody N-2 variable region
EVQLKESGGGLVKPGGSLKLSCAASGFTFSDYGMHWVRQAPEKGLEWVAYISSGSSTIYYADTVKGRFTISRDNAKNTLFLQMTSLRSEDTAIYYCARLDDYDADYYAMDYWGQGTSVTVSS

SEQ ID NO: 65 - protein, 122 aa, Mus musculus
  DOMAIN (1)..(122): Amino acid sequence of coronavirus N protein antigen-specific IgG2c heavy chain antibody N-3 variable region
QVQLKESGPGLVKPSQSLSLTCTVTGYSITSGYDWHWIRHFPGNKLEWMGYISYSGSTNYNPSLKSRISITHDTSKNHFFLKLNSVTTEDTATYYCARGDDYDGDYYTMDYWGQGTSVTVSS

SEQ ID NO: 66 - protein, 122 aa, Mus musculus
  DOMAIN (1)..(122): Amino acid sequence of coronavirus N protein antigen-specific IgG2c heavy chain antibody N-5 variable region
EVQLKESGPGLVKPSQSLSLTCSVTGYSITSGYYWYWIRQFPGNKQEWLGYITYDGSNHYNPSLKNRISITRDTSKNQFFLKLSSVTTEDTATYYCARGDDYDGDYYTMDYWGQGTSVTVSS

SEQ ID NO: 67 - protein, 116 aa, Mus musculus
  DOMAIN (1)..(116): Amino acid sequence of coronavirus N protein antigen-specific IgG2c heavy chain antibody N-23 variable region
EVQLQESGGGLVKPGGSLKLSCAASGFTFSDYGMHWVRQAPEKGLEWVAYISSGSSTIYYADTVKGRFTISRDNAKNTLFLQMTSLRSEDTAMYYCARGLDAMDNWGQGTSVTVSS

SEQ ID NO: 68 - DNA, 18 bp, Artificial sequence
  PCR forward primer JH2, for amplifying mu gene
  misc_feature (1)..(18)
ctactggggccaaggcac

SEQ ID NO: 69 - DNA, 20 bp, Artificial sequence
  PCR reverse primer q-IgM-CH1-R, for amplifying mu gene
  misc_feature (1)..(20)
agcccatggccaccagattc

SEQ ID NO: 70 - DNA, 22 bp, Artificial sequence
  PCR forward primer q-IgG2c-hinge-CH2-F, for amplifying gamma2c gene
  misc_feature (1)..(22)
atgcgcagctccagacctcttg

SEQ ID NO: 71 - DNA, 19 bp, Artificial sequence
  PCR reverse primer q-IgG2c-CH2-R, for amplifying gamma2c gene
  misc_feature (1)..(19)
ggctcagggagatcatgag

SEQ ID NO: 72 - DNA, 22 bp, Artificial sequence
  PCR forward primer JH2-3, for amplifying alpha gene
  misc_feature (1)..(22)
tactggggccaaggcaccactc

SEQ ID NO: 73 - DNA, 22 bp, Artificial sequence
  PCR reverse primer q-IgA-CH1-R, for amplifying alpha gene
  misc_feature (1)..(22)
gggtcacttgacagagctcgtg

SEQ ID NO: 74 - DNA, 20 bp, Artificial Sequence
  Primer Ighg-1F
  misc_feature (1)..(20)
ggaatcaaaggacagcagga

SEQ ID NO: 75 - DNA, 20 bp, Artificial Sequence
  Primer Ighg-1R
agtgtcaccgaggatccaga

SEQ ID NO: 76 - DNA, 20 bp, Artificial Sequence
  Primer Ighg-2R
  misc_feature (1)..(20)
ccaaacagggcttggagact